European Patent Application EP 4 151 650 A1, published March 22, 2023. Title: Monoclonal Antibody against Human Activated Protein C and Preparation and Use Thereof. Applicant: Shanghai RAAS blood products Co., Ltd. The sequence listing filed with the application follows.

SEQUENCE LISTING (92 sequences)

SEQ ID NO: 1 - protein, 118 aa, Artificial Sequence
EVQLVESGGGLVQPGGSLRLSCAASGFTFSNYYLNWVRQAPGKGLEWVGDIRLKSNNYEKHYAESVKGRFTISRDDSKSITYLQMNSLRAEDTAVYYCAREGDYFDYWGQGTTVTVSS

SEQ ID NO: 2 - protein, 111 aa, Artificial Sequence
DIQMTQSPSSLSASVGDRVTITCRASESVDSFGATFMHWYQQKPGKAPKLLIYLASNLESGVPSRFSGSGSGTDFTLTISSLQPEDFATYYCQQNNEDPYTFGQGTKLEIK

SEQ ID NO: 3 - protein, 118 aa, Artificial Sequence; identical to SEQ ID NO: 1

SEQ ID NO: 4 - protein, 111 aa, Artificial Sequence
NIVLTQSPSSLSASVGDRVTITCRASESVDSFGATFMHWYQQKPGKPPKLLIYLASNLESGVPSRFSGSGSRTDFTLTISSLQPEDFATYYCQQNNEDPYTFGQGTKLEIK

SEQ ID NO: 5 - protein, 118 aa, Artificial Sequence; identical to SEQ ID NO: 1

SEQ ID NO: 6 - protein, 111 aa, Artificial Sequence
DIQLTQSPSSLSASVGDRVTITCRASESVDSFGATFMHWYQQKPGKAPKLLIYLASNLESGVPSRFSGSGSGTDFTLTISSLQPEDFATYYCQQNNEDPYTFGQGTKLEIK

SEQ ID NO: 7 - protein, 118 aa, Artificial Sequence
EVQLVESGGGLVQPGGSLRLSCAASGFTFSFYYLNWVRQAPGKGLEWVGDIRLKSNNYEKHYAESVKGRFTISRDDSKSITYLQMNSLRAEDTAVYYCAREGDYFDYWGQGTTVTVSS

SEQ ID NO: 8 - protein, 111 aa, Artificial Sequence
DIQLTQSPSSLSASVGDRVTITCRASESVDSFGATFMHWYQQKPGKAPKLLIYLASWLGSGVPSRFSGSGSGTDFTLTISSLQPEDFATYYCQQNNEDPYTFGQGTKLEIK

SEQ ID NO: 9 - protein, 118 aa, Artificial Sequence
EVQLVESGGGLVQPGGSLRLSCAASGFTFSFYYLNWVRQAPGKGLEWVGDIRLKKNNYEKHYAESVKGRFTISRDDSKSITYLQMNSLRAEDTAVYYCAREGDYFDYWGQGTTVTVSS

SEQ ID NO: 10 - protein, 111 aa, Artificial Sequence
DIQLTQSPSSLSASVGDRVTITCRASESVDSFGATFMHWYQQKPGKAPKLLIYLASWLESGVPSRFSGSGSGTDFTLTISSLQPEDFATYYCVQNNEDPYTFGQGTKLEIK

SEQ ID NO: 11 - protein, 118 aa, Artificial Sequence; identical to SEQ ID NO: 9

SEQ ID NO: 12 - protein, 111 aa, Artificial Sequence
DIQLTQSPSSLSASVGDRVTITCRASESVDSFGATFMHWYQQKPGKAPKLLIYLASRLGSGVPSRFSGSGSGTDFTLTISSLQPEDFATYYCVQNNEDPYTFGQGTKLEIK

SEQ ID NO: 13 - protein, 118 aa, Artificial Sequence; identical to SEQ ID NO: 7

SEQ ID NO: 14 - protein, 111 aa, Artificial Sequence; identical to SEQ ID NO: 12

SEQ ID NO: 15 - protein, 118 aa, Artificial Sequence; identical to SEQ ID NO: 9

SEQ ID NO: 16 - protein, 111 aa, Artificial Sequence
DIQLTQSPSSLSASVGDRVTITCRASESVDSFGATFMHWYQQKPGKAPKLLIYLASWLGSGVPSRFSGSGSGTDFTLTISSLQPEDFATYYCVQNNEDPYTFGQGTKLEIK

SEQ ID NO: 17 - protein, 118 aa, Artificial Sequence; identical to SEQ ID NO: 9

SEQ ID NO: 18 - protein, 111 aa, Artificial Sequence
DIQLTQSPSSLSASVGDRVTITCRASESVDSFGATFMHWYQQKPGKAPKLLIYLASRLGSGVPSRFSGSGSGTDFTLTISSLQPEDFATYYCQQNNEDPYTFGQGTKLEIK

SEQ ID NO: 19 - protein, 118 aa, Artificial Sequence; identical to SEQ ID NO: 7

SEQ ID NO: 20 - protein, 111 aa, Artificial Sequence
DIQLTQSPSSLSASVGDRVTITCRASESVDSFGATFMHWYQQKPGKAPKLLIYLASRLESGVPSRFSGSGSGTDFTLTISSLQPEDFATYYCQQNNEDPYTFGQGTKLEIK

SEQ ID NO: 21 - protein, 118 aa, Artificial Sequence
EVQLVESGGGLVQPGGSLRLSCAASGFTFSFYYLNWVRQAPGKGLEWVGDIRLKKNNYEKHYAESVKGRFTISRDDSKSITYLQMNSLRAEDTAVYYCAREGDTFDYWGQGTTVTVSS

SEQ ID NO: 22 - protein, 111 aa, Artificial Sequence; identical to SEQ ID NO: 12

SEQ ID NO: 23 - protein, 118 aa, Artificial Sequence; identical to SEQ ID NO: 21

SEQ ID NO: 24 - protein, 111 aa, Artificial Sequence; identical to SEQ ID NO: 18

SEQ ID NO: 25 - protein, 118 aa, Artificial Sequence
EVQLVESGGGLVQPGGSLRLSCAASGFTFSNYYLNWVRQAPGKGLEWVGDIRLKKNNYEKHYAESVKGRFTISRDDSKSITYLQMNSLRAEDTAVYYCAREGDTFDYWGQGTTVTVSS

SEQ ID NO: 26 - protein, 111 aa, Artificial Sequence; identical to SEQ ID NO: 12

SEQ ID NO: 27 - protein, 5 aa, Artificial Sequence
NYYLN

SEQ ID NO: 28 - protein, 19 aa, Artificial Sequence
DIRLKSNNYEKHYAESVKG

SEQ ID NO: 29 - protein, 7 aa, Artificial Sequence
EGDYFDY

SEQ ID NO: 30 - protein, 15 aa, Artificial Sequence
RASESVDSFGATFMH

SEQ ID NO: 31 - protein, 7 aa, Artificial Sequence
LASNLES

SEQ ID NO: 32 - protein, 9 aa, Artificial Sequence
QQNNEDPYT

SEQ ID NO: 33 - protein, 5 aa, Artificial Sequence
FYYLN

SEQ ID NO: 34 - protein, 19 aa, Artificial Sequence
DIRLKSNNYEKHYAESVKG

SEQ ID NO: 35 - protein, 7 aa, Artificial Sequence
EGDYFDY

SEQ ID NO: 36 - protein, 15 aa, Artificial Sequence
RASESVDSFGATFMH

SEQ ID NO: 37 - protein, 7 aa, Artificial Sequence
LASWLGS

SEQ ID NO: 38 - protein, 9 aa, Artificial Sequence
QQNNEDPYT

SEQ ID NO: 39 - protein, 5 aa, Artificial Sequence
FYYLN

SEQ ID NO: 40 - protein, 19 aa, Artificial Sequence
DIRLKKNNYEKHYAESVKG

SEQ ID NO: 41 - protein, 7 aa, Artificial Sequence
EGDYFDY

SEQ ID NO: 42 - protein, 15 aa, Artificial Sequence
RASESVDSFGATFMH

SEQ ID NO: 43 - protein, 7 aa, Artificial Sequence
LASWLES

SEQ ID NO: 44 - protein, 9 aa, Artificial Sequence
VQNNEDPYT

SEQ ID NO: 45 - protein, 5 aa, Artificial Sequence
FYYLN

SEQ ID NO: 46 - protein, 19 aa, Artificial Sequence
DIRLKKNNYEKHYAESVKG

SEQ ID NO: 47 - protein, 7 aa, Artificial Sequence
EGDYFDY

SEQ ID NO: 48 - protein, 15 aa, Artificial Sequence
RASESVDSFGATFMH

SEQ ID NO: 49 - protein, 7 aa, Artificial Sequence
LASRLGS

SEQ ID NO: 50 - protein, 9 aa, Artificial Sequence
VQNNEDPYT

SEQ ID NO: 51 - protein, 5 aa, Artificial Sequence
FYYLN

SEQ ID NO: 52 - protein, 19 aa, Artificial Sequence
DIRLKSNNYEKHYAESVKG

SEQ ID NO: 53 - protein, 7 aa, Artificial Sequence
EGDYFDY

SEQ ID NO: 54 - protein, 15 aa, Artificial Sequence
RASESVDSFGATFMH

SEQ ID NO: 55 - protein, 7 aa, Artificial Sequence
LASRLGS

SEQ ID NO: 56 - protein, 9 aa, Artificial Sequence
VQNNEDPYT

SEQ ID NO: 57 - protein, 5 aa, Artificial Sequence
FYYLN

SEQ ID NO: 58 - protein, 19 aa, Artificial Sequence
DIRLKKNNYEKHYAESVKG

SEQ ID NO: 59 - protein, 7 aa, Artificial Sequence
EGDYFDY

SEQ ID NO: 60 - protein, 15 aa, Artificial Sequence
RASESVDSFGATFMH

SEQ ID NO: 61 - protein, 7 aa, Artificial Sequence
LASWLGS

SEQ ID NO: 62 - protein, 9 aa, Artificial Sequence
VQNNEDPYT

SEQ ID NO: 63 - protein, 5 aa, Artificial Sequence
FYYLN

SEQ ID NO: 64 - protein, 19 aa, Artificial Sequence
DIRLKKNNYEKHYAESVKG

SEQ ID NO: 65 - protein, 7 aa, Artificial Sequence
EGDYFDY

SEQ ID NO: 66 - protein, 15 aa, Artificial Sequence
RASESVDSFGATFMH

SEQ ID NO: 67 - protein, 7 aa, Artificial Sequence
LASRLGS

SEQ ID NO: 68 - protein, 9 aa, Artificial Sequence
QQNNEDPYT

SEQ ID NO: 69 - protein, 5 aa, Artificial Sequence
FYYLN

SEQ ID NO: 70 - protein, 19 aa, Artificial Sequence
DIRLKSNNYEKHYAESVKG

SEQ ID NO: 71 - protein, 7 aa, Artificial Sequence
EGDYFDY

SEQ ID NO: 72 - protein, 15 aa, Artificial Sequence
RASESVDSFGATFMH

SEQ ID NO: 73 - protein, 7 aa, Artificial Sequence
LASRLES

SEQ ID NO: 74 - protein, 9 aa, Artificial Sequence
QQNNEDPYT

SEQ ID NO: 75 - protein, 5 aa, Artificial Sequence
FYYLN

SEQ ID NO: 76 - protein, 19 aa, Artificial Sequence
DIRLKKNNYEKHYAESVKG

SEQ ID NO: 77 - protein, 7 aa, Artificial Sequence
EGDTFDY

SEQ ID NO: 78 - protein, 15 aa, Artificial Sequence
RASESVDSFGATFMH

SEQ ID NO: 79 - protein, 7 aa, Artificial Sequence
LASRLGS

SEQ ID NO: 80 - protein, 9 aa, Artificial Sequence
VQNNEDPYT

SEQ ID NO: 81 - protein, 5 aa, Artificial Sequence
FYYLN

SEQ ID NO: 82 - protein, 19 aa, Artificial Sequence
DIRLKKNNYEKHYAESVKG

SEQ ID NO: 83 - protein, 7 aa, Artificial Sequence
EGDTFDY

SEQ ID NO: 84 - protein, 15 aa, Artificial Sequence
RASESVDSFGATFMH

SEQ ID NO: 85 - protein, 7 aa, Artificial Sequence
LASRLGS

SEQ ID NO: 86 - protein, 9 aa, Artificial Sequence
QQNNEDPYT

SEQ ID NO: 87 - protein, 5 aa, Artificial Sequence
NYYLN

SEQ ID NO: 88 - protein, 19 aa, Artificial Sequence
DIRLKKNNYEKHYAESVKG

SEQ ID NO: 89 - protein, 7 aa, Artificial Sequence
EGDTFDY

SEQ ID NO: 90 - protein, 15 aa, Artificial Sequence
RASESVDSFGATFMH

SEQ ID NO: 91 - protein, 15 aa, Artificial Sequence
RASESVDSFGATFMH

SEQ ID NO: 92 - protein, 9 aa, Artificial Sequence
VQNNEDPYT